European Patent Application EP 4 674 870 A1, published January 7, 2026. Title: ANTI-TL1A ANTIBODY, PREPARATION METHOD THEREFOR AND USE THEREOF. Applicant: SUNSHINE GUOJIAN PHARMACEUTICAL (SHANGHAI) CO., LTD. Application EP. The sequence listing filed with the application follows.

SEQUENCE LISTING (48 sequences)

SEQ ID NO: 1 - protein, 180 aa, Homo sapiens
LKGQEFAPSHQQVYAPLRADGDKPRAHLTVVRQTPTQHFKNQFPALHWEHELGLAFTKNRMNYTNKFLLIPESGDYFIYSQVTFRGMTSECSEIRQAGRPNKPDSITVVITKVTDSYPEPTQLLMGTKSVCEVGSNWFQPIYLGAMFSLQEGDKLMVNVSDISLVDYTKEDKTFFGAFLL

SEQ ID NO: 2 - DNA, 357 bp, synthetic construct
  source 1..357: mol_type = other DNA; note = Nucleotide sequence of the heavy chain variable region of 728H4D9
gaggtccagctgcaacagtctggacctgagctggtgaagcctggagcttcaatgaagatatcctgcaaggcttctggttactcattcactggctacaccatgaactgggtgaagcagagccatggaaagaaccttgagtggattggacttattaatccttacagcggtggtactaactacaaccagaagttcaagggcaaggccacattaactgtagacaagacatccagcacagcctacatggagctcctcagtctgacatctgaggactctgcagtctattactgtgcgtccatctaccaaaggcacgacgggattgcttactggggccaagggactctggtcactgtctctgca

SEQ ID NO: 3 - protein, 119 aa, synthetic construct
  source 1..119: note = Amino acid sequence of the heavy chain variable region of 728H4D9
EVQLQQSGPELVKPGASMKISCKASGYSFTGYTMNWVKQSHGKNLEWIGLINPYSGGTNYNQKFKGKATLTVDKTSSTAYMELLSLTSEDSAVYYCASIYQRHDGIAYWGQGTLVTVSA

SEQ ID NO: 4 - DNA, 318 bp, synthetic construct
  source 1..318: mol_type = other DNA; note = Nucleotide sequence of the light chain variable region of 728H4D9
caaattgttctcacccagtctccagcaatcatgtctgcatctccaggggagaaggtcaccatgacctgcagtgccagctcaagtgtaaattacatgcactggtaccagcagaagtcaggcacctcccccaaaagatggatttatgacacatccaaactggcttctggagtcccaactcgcttcagtggcagtgggtctgggacctcttactctctcacaatcagcagcatggaggctgaagatgctgccacttattactgccagcagtggagtagtagcccatacacgttcggaggggggaccaagctggaaatcaaa

SEQ ID NO: 5 - protein, 106 aa, synthetic construct
  source 1..106: note = Amino acid sequence of the light chain variable region of 728H4D9
QIVLTQSPAIMSASPGEKVTMTCSASSSVNYMHWYQQKSGTSPKRWIYDTSKLASGVPTRFSGSGSGTSYSLTISSMEAEDAATYYCQQWSSSPYTFGGGTKLEIK

SEQ ID NO: 6 - DNA, 357 bp, synthetic construct
  source 1..357: mol_type = other DNA; note = Nucleotide sequence of the heavy chain variable region of 311C9E10
gaagtgaaacttgaggagtctggaggaggcttagtgcaacctggaggatccatgaaactctcctgtgttgcctctggattcactttcagtaactactggatgaactgggtccgccagtctccagagaaggggcttgagtgggttgctggaattagattgaaatctaataattatacaacacagtatgcggagtctgtgaaagggaggttcaccatttcaagagatgattccaaaagtagtgtctacctgcaaatgaacaacttaagagctgaagacactggcatttattattgtaccccattactcctcaatggtatggactactggggtcaaggaacctcagtcaccgtctcctca

SEQ ID NO: 7 - protein, 119 aa, synthetic construct
  source 1..119: note = Amino acid sequence of the heavy chain variable region of 311C9E10
EVKLEESGGGLVQPGGSMKLSCVASGFTFSNYWMNWVRQSPEKGLEWVAGIRLKSNNYTTQYAESVKGRFTISRDDSKSSVYLQMNNLRAEDTGIYYCTPLLLNGMDYWGQGTSVTVSS

SEQ ID NO: 8 - DNA, 318 bp, synthetic construct
  source 1..318: mol_type = other DNA; note = Nucleotide sequence of the light chain variable region of 311C9E10
gaaaatgttctcacccagtctccagcaatcatgtctgcatctccaggggaaaaggtcatcatgacctgtagtgccagctcaagtgtaagctacatgcactggtaccagcggaagtcaaacacctcccccaaactctggatttatgacacatccaatctggcttctggagtcccaggtcgcttcagtggcactgggtctggaaactcttactctctcacgatcagcagcatggaggctgaagatgttgccacttattactgttttcaggagagtgggtacccattcacgttcggctcggggacaaagttggaaataaaa

SEQ ID NO: 9 - protein, 106 aa, synthetic construct
  source 1..106: note = Amino acid sequence of the light chain variable region of 311C9E10
ENVLTQSPAIMSASPGEKVIMTCSASSSVSYMHWYQRKSNTSPKLWIYDTSNLASGVPGRFSGTGSGNSYSLTISSMEAEDVATYYCFQESGYPFTFGSGTKLEIK

SEQ ID NO: 10 - protein, 5 aa, synthetic construct
  source 1..5: note = 728H4D9 HCDR1
GYTMN

SEQ ID NO: 11 - protein, 17 aa, synthetic construct
  source 1..17: note = 728H4D9 HCDR2
LINPYSGGTNYNQKFKG

SEQ ID NO: 12 - protein, 10 aa, synthetic construct
  source 1..10: note = 728H4D9 HCDR3
IYQRHDGIAY

SEQ ID NO: 13 - protein, 10 aa, synthetic construct
  source 1..10: note = 728H4D9 LCDR1
SASSSVNYMH

SEQ ID NO: 14 - protein, 7 aa, synthetic construct
  source 1..7: note = 728H4D9 LCDR2
DTSKLAS

SEQ ID NO: 15 - protein, 9 aa, synthetic construct
  source 1..9: note = 728H4D9 LCDR3
QQWSSSPYT

SEQ ID NO: 16 - protein, 119 aa, synthetic construct
  source 1..119: note = Amino acid sequence of the heavy chain variable region of humanized antibody 72851
QVQLVQSGAEVKKPGASVKVSCKASGYSFTGYTMNWVRQAPGQNLEWIGLINPYSGGTNYNQKFKGRATLTVDTSISTAYMELSRLRSDDTAVYYCASIYQRHDGIAYWGQGTLVTVSS

SEQ ID NO: 17 - protein, 106 aa, synthetic construct
  source 1..106: note = Amino acid sequence of the light chain variable region of humanized antibody 72851
EIVLTQSPDFQSVTPKEKVTITCSASSSVNYMHWYQQKPDQSPKLLIKDTSKLASGVPSRFSGSGSGTDFTLTINSLEAEDAATYYCQQWSSSPYTFGGGTKVEIK

SEQ ID NO: 18 - protein, 5 aa, synthetic construct
  source 1..5: note = 311C9E10/311V25/311V31/311V34/311V25-7/311V31-7/311V34-7 HCDR1
NYWMN

SEQ ID NO: 19 - protein, 19 aa, synthetic construct
  source 1..19: note = 311C9E10 HCDR2
GIRLKSNNYTTQYAESVKG

SEQ ID NO: 20 - protein, 8 aa, synthetic construct
  source 1..8: note = 311C9E10/311V25/311V31/311V34 HCDR3
LLLNGMDY

SEQ ID NO: 21 - protein, 10 aa, synthetic construct
  source 1..10: note = 311C9E10 LCDR1
SASSSVSYMH

SEQ ID NO: 22 - protein, 7 aa, synthetic construct
  source 1..7: note = 311C9E10 LCDR2
DTSNLAS

SEQ ID NO: 23 - protein, 9 aa, synthetic construct
  source 1..9: note = 311C9E10 LCDR3
FQESGYPFT

SEQ ID NO: 24 - protein, 119 aa, synthetic construct
  source 1..119: note = Amino acid sequence of the heavy chain variable region of humanized antibody 31122
EVQLVESGGGLVQPGGSLKLSCAASGFTFSNYWMNWVRQASGKGLEWVGGIRLKSNNYTTQYAESVKGRFTISRDDSKNTAYLQMNSLKTEDTAVYYCTPLLLNGMDYWGQGTTVTVSS

SEQ ID NO: 25 - protein, 106 aa, synthetic construct
  source 1..106: note = Amino acid sequence of the light chain variable region of humanized antibody 31122
EIVLTQSPDFQSVTPKEKVTITCSASSSVSYMHWYQQKPDQSPKLWIYDTSNLASGVPSRFSGSGSGTDFTLTINSLEAEDAATYYCFQESGYPFTFGQGTKLEIK

SEQ ID NO: 26 - protein, 119 aa, synthetic construct
  source 1..119: note = 311V25-HC amino acid sequence
EVQLVESGGGLVQPGGSLKLSCAASGFTFSNYWMNWVRQASGKGLEWVGGIRLKSNNYATQYAESVKGRFTISRDDSKNTAYLQMNSLKTEDTAVYYCTPLLLNGMDYWGQGTTVTVSS

SEQ ID NO: 27 - protein, 119 aa, synthetic construct
  source 1..119: note = 311V31-HC amino acid sequence
EVQLVESGGGLVQPGGSLKLSCAASGFTFSNYWMNWVRQASGKGLEWVGGIRLKSNNYKTQYAESVKGRFTISRDDSKNTAYLQMNSLKTEDTAVYYCTPLLLNGMDYWGQGTTVTVSS

SEQ ID NO: 28 - protein, 119 aa, synthetic construct
  source 1..119: note = 311V34-HC amino acid sequence
EVQLVESGGGLVQPGGSLKLSCAASGFTFSNYWMNWVRQASGKGLEWVGGIRLKSNNYRTQYAESVKGRFTISRDDSKNTAYLQMNSLKTEDTAVYYCTPLLLNGMDYWGQGTTVTVSS

SEQ ID NO: 29 - protein, 119 aa, synthetic construct
  source 1..119: note = 311V25-7-HC amino acid sequence
EVQLVESGGGLVQPGGSLKLSCAASGFTFSNYWMNWVRQASGKGLEWVGGIRLKSNNYATQYAESVKGRFTISRDDSKNTAYLQMNSLKTEDTAVYYCTPLLLSGMDYWGQGTTVTVSS

SEQ ID NO: 30 - protein, 119 aa, synthetic construct
  source 1..119: note = 311V31-7-HC amino acid sequence
EVQLVESGGGLVQPGGSLKLSCAASGFTFSNYWMNWVRQASGKGLEWVGGIRLKSNNYKTQYAESVKGRFTISRDDSKNTAYLQMNSLKTEDTAVYYCTPLLLSGMDYWGQGTTVTVSS

SEQ ID NO: 31 - protein, 119 aa, synthetic construct
  source 1..119: note = 311V34-7-HC amino acid sequence
EVQLVESGGGLVQPGGSLKLSCAASGFTFSNYWMNWVRQASGKGLEWVGGIRLKSNNYRTQYAESVKGRFTISRDDSKNTAYLQMNSLKTEDTAVYYCTPLLLSGMDYWGQGTTVTVSS

SEQ ID NO: 32 - protein, 417 aa, Homo sapiens
MEQRPRGCAAVAAALLLVLLGARAQGGTRSPRCDCAGDFHKKIGLFCCRGCPAGHYLKAPCTEPCGNSTCLVCPQDTFLAWENHHNSECARCQACDEQASQVALENCSAVADTRCGCKPGWFVECQVSQCVSSSPFYCQPCLDCGALHRHTRLLCSRRDTDCGTCLPGFYEHGDGCVSCPTSTLGSCPERCAAVCGWRQMFWVQVLLAGLVVPLLLGATLTYTYRHCWPHKPLVTADEAGMEALTPPPATHLSPLDSAHTLLAPPDSSEKICTVQLVGNSWTPGYPETQEALCPQVTWSWDQLPSRALGPAAAPTLSPESPAGSPAMMLQPGPQLYDVMDAVPARRWKEFVRTLGLREAEIEAVEVEIGRFRDQQYEMLKRWRQQQPAGLGAVYAALERMGLDGCVEDLRSRLQRGP

SEQ ID NO: 33 - protein, 330 aa, Homo sapiens
ASTKGPSVFPLAPSSKSTSGGTAALGCLVKDYFPEPVTVSWNSGALTSGVHTFPAVLQSSGLYSLSSVVTVPSSSLGTQTYICNVNHKPSNTKVDKKVEPKSCDKTHTCPPCPAPEAAGGPSVFLFPPKPKDTLYITREPEVTCVVVDVSHEDPEVKFNWYVDGVEVHNAKTKPREEQYNSTYRVVSVLTVLHQDWLNGKEYKCKVSNKALPAPIEKTISKAKGQPREPQVYTLPPSREEMTKNQVSLTCLVKGFYPSDIAVEWESNGQPENNYKTTPPVLDSDGSFFLYSKLTVDKSRWQQGNVFSCSVMHEALHNHYTQKSLSLSPGK

SEQ ID NO: 34 - protein, 107 aa, Homo sapiens [sequence omitted]

SEQ ID NO: 35 - DNA, 357 bp, synthetic construct
  source 1..357: mol_type = other DNA; note = Nucleotide sequence of the heavy chain variable region of humanized antibody 72851
caagtgcagctggtgcagagcggcgccgaggtgaagaagcctggcgctagcgtgaaggtgagctgcaaggctagcggctacagcttcaccggctacaccatgaactgggtgagacaagcccctggacagaacctggagtggatcggcctgatcaacccttacagcggcggaaccaactacaatcagaagttcaagggcagagccacactgaccgtggacacaagcatcagcaccgcctacatggagctgagcagactgagaagcgacgacaccgccgtgtattattgcgcctccatctatcagagacacgacggcatcgcctactggggccaaggcaccctggtgaccgtgagcagc

SEQ ID NO: 36 - DNA, 318 bp, synthetic construct
  source 1..318: mol_type = other DNA; note = Nucleotide sequence of the light chain variable region of humanized antibody 72851
gagatcgtgctgacacagagccctgactttcagagcgtgacccctaaggagaaggtgaccattacctgcagcgctagcagcagcgtgaactacatgcactggtatcagcagaagcctgatcagagccctaagctgctgatcaaggacacaagcaagctggctagcggcgtgcctagcagattcagcggcagcggcagcggcaccgacttcaccctgaccatcaacagcctggaggccgaggacgccgccacctactactgtcagcagtggagcagcagcccttacaccttcggcggaggcaccaaggtggagatcaaa

SEQ ID NO: 37 - DNA, 357 bp, synthetic construct
  source 1..357: mol_type = other DNA; note = Nucleotide sequence of the heavy chain variable region of humanized antibody 31122
gaggtgcagctggtcgagtccggaggcggactggtccaacctggcggaagcctgaagctgagctgcgccgctagcggcttcaccttcagcaactactggatgaactgggtgagacaagctagcggcaagggcctggagtgggtgggcggcatcagactgaagagcaacaactacaccacacagtacgccgagagcgtgaagggcagattcaccatcagcagagacgacagcaagaacaccgcctacctgcagatgaacagcctgaagaccgaggacaccgccgtgtactactgcacacctctgctcctgaacggcatggactactggggccaaggcaccaccgtgaccgtgagcagc

SEQ ID NO: 38 - DNA, 318 bp, synthetic construct
  source 1..318: mol_type = other DNA; note = Nucleotide sequence of the light chain variable region of humanized antibody 31122
gagatcgtgctgacacagagccctgactttcagagcgtgacccctaaggagaaggtgaccatcacctgcagcgctagcagcagcgtgagctacatgcactggtatcagcagaagcctgatcagagccctaagctgtggatctacgacacaagcaacctggctagcggcgtgcctagcagattcagcggcagcggcagcggcaccgacttcaccctgaccatcaacagcctggaggccgaggacgccgccacctactactgcttccaagagagcggctaccctttcaccttcggccaaggcaccaagctggagatcaaa

SEQ ID NO: 39 - protein, 19 aa, synthetic construct
  source 1..19: note = 311V25/311V25-7 HCDR2
GIRLKSNNYATQYAESVKG

SEQ ID NO: 40 - protein, 19 aa, synthetic construct
  source 1..19: note = 311V31/311V31-7 HCDR2
GIRLKSNNYKTQYAESVKG

SEQ ID NO: 41 - protein, 19 aa, synthetic construct
  source 1..19: note = 311V34/311V34-7 HCDR2
GIRLKSNNYRTQYAESVKG

SEQ ID NO: 42 - protein, 8 aa, synthetic construct
  source 1..8: note = 311V25-7/311V31-7/311V34-7 HCDR3
LLLSGMDY

SEQ ID NO: 43 - DNA, 357 bp, synthetic construct
  source 1..357: mol_type = other DNA; note = 311V25-HC nucleotide sequence
gaggtgcagctggtcgagtccggaggcggactggtccaacctggcggaagcctgaagctgagctgcgccgctagcggcttcaccttcagcaactactggatgaactgggtgagacaagctagcggcaagggcctggagtgggtgggcggcatcagactgaagagcaacaactacgccacacagtacgccgagagcgtgaagggcagattcaccatcagcagagacgacagcaagaacaccgcctacctgcagatgaacagcctgaagaccgaggacaccgccgtgtactactgcacacctctgctcctgaacggcatggactactggggccaaggcaccaccgtgaccgtgagcagc

SEQ ID NO: 44 - DNA, 357 bp, synthetic construct
  source 1..357: mol_type = other DNA; note = 311V31-HC nucleotide sequence
gaggtgcagctggtcgagtccggaggcggactggtccaacctggcggaagcctgaagctgagctgcgccgctagcggcttcaccttcagcaactactggatgaactgggtgagacaagctagcggcaagggcctggagtgggtgggcggcatcagactgaagagcaacaactacaagacacagtacgccgagagcgtgaagggcagattcaccatcagcagagacgacagcaagaacaccgcctacctgcagatgaacagcctgaagaccgaggacaccgccgtgtactactgcacacctctgctcctgaacggcatggactactggggccaaggcaccaccgtgaccgtgagcagc

SEQ ID NO: 45 - DNA, 357 bp, synthetic construct
  source 1..357: mol_type = other DNA; note = 311V34-HC nucleotide sequence
gaggtgcagctggtcgagtccggaggcggactggtccaacctggcggaagcctgaagctgagctgcgccgctagcggcttcaccttcagcaactactggatgaactgggtgagacaagctagcggcaagggcctggagtgggtgggcggcatcagactgaagagcaacaactacagaacacagtacgccgagagcgtgaagggcagattcaccatcagcagagacgacagcaagaacaccgcctacctgcagatgaacagcctgaagaccgaggacaccgccgtgtactactgcacacctctgctcctgaacggcatggactactggggccaaggcaccaccgtgaccgtgagcagc

SEQ ID NO: 46 - DNA, 357 bp, synthetic construct
  source 1..357: mol_type = other DNA; note = 311V25-7-HC nucleotide sequence
gaggtgcagctggtcgagtccggaggcggactggtccaacctggcggaagcctgaagctgagctgcgccgctagcggcttcaccttcagcaactactggatgaactgggtgagacaagctagcggcaagggcctggagtgggtgggcggcatcagactgaagagcaacaactacgccacacagtacgccgagagcgtgaagggcagattcaccatcagcagagacgacagcaagaacaccgcctacctgcagatgaacagcctgaagaccgaggacaccgccgtgtactactgcacacctctgctcctgagcggcatggactactggggccaaggcaccaccgtgaccgtgagcagc

SEQ ID NO: 47 - DNA, 357 bp, synthetic construct
  source 1..357: mol_type = other DNA; note = 311V31-7-HC nucleotide sequence
gaggtgcagctggtcgagtccggaggcggactggtccaacctggcggaagcctgaagctgagctgcgccgctagcggcttcaccttcagcaactactggatgaactgggtgagacaagctagcggcaagggcctggagtgggtgggcggcatcagactgaagagcaacaactacaagacacagtacgccgagagcgtgaagggcagattcaccatcagcagagacgacagcaagaacaccgcctacctgcagatgaacagcctgaagaccgaggacaccgccgtgtactactgcacacctctgctcctgagcggcatggactactggggccaaggcaccaccgtgaccgtgagcagc

SEQ ID NO: 48 - DNA, 357 bp, synthetic construct
  source 1..357: mol_type = other DNA; note = 311V34-7-HC nucleotide sequence
gaggtgcagctggtcgagtccggaggcggactggtccaacctggcggaagcctgaagctgagctgcgccgctagcggcttcaccttcagcaactactggatgaactgggtgagacaagctagcggcaagggcctggagtgggtgggcggcatcagactgaagagcaacaactacagaacacagtacgccgagagcgtgaagggcagattcaccatcagcagagacgacagcaagaacaccgcctacctgcagatgaacagcctgaagaccgaggacaccgccgtgtactactgcacacctctgctcctgagcggcatggactactggggccaaggcaccaccgtgaccgtgagcagc